European Patent Application EP 4 137 121 A1, published February 22, 2023. Title: PHARMACEUTICAL COMPOSITION COMPRISING NANOPARTICLES FOR THE TARGETED DELIVERY OF ANTIGENS. Applicant: TOPAS THERAPEUTICS GMBH. The sequence listing filed with the application follows.

SEQUENCE LISTING (4 sequences)

SEQ ID NO: 1 - protein, 15 aa, Artificial Sequence
  antigenic peptide
LNSKIAFKIVSQEPA

SEQ ID NO: 2 - protein, 15 aa, Artificial Sequence
  antigenic peptide
TPMFLLSRNTGEVRT

SEQ ID NO: 3 - protein, 15 aa, Artificial Sequence
  antigenic peptide
NIKVKDVNDNFPMFR

SEQ ID NO: 4 - protein, 15 aa, Artificial Sequence
  antigenic peptide
REGIAFRPASKTFTV